European Patent Application EP 4 506 453 A1, published February 12, 2025. Title: Bst DNA polymerase, reagent composition and method for amplifying nucleic acid. Applicant: SYSMEX CORPORATION. Application JP. The sequence listing filed with the application follows.

SEQUENCE LISTING (9 sequences)

SEQ ID NO: 1 - protein, 587 aa, Geobacillus stearothermophilus
AEGEKPLEEMEFAIVDVITEEMLADKAALVVEVMEENYHDAPIVGIALVNEHGRFFMRPETALADSQFLAWLADETKKKSMFDAKRAVVALKWKGIELRGVAFDLLLAAYLLNPAQDAGDIAAVAKMKQYEAVRSDEAVYGKGVKRSLPDEQTLAEHLVRKAAAIWALEQPFMDDLRNNEQDQLLTKLEQPLAAILAEMEFTGVNVDTKRLEQMGSELAEQLRAIEQRIYELAGQEFNINSPKQLGVILFEKLQLPVLKKTKTGYSTSADVLEKLAPHHEIVENILHYRQLGKLQSTYIEGLLKVVRPDTGKVHTMFNQALTQTGRLSSAEPNLQNIPIRLEEGRKIRQAFVPSEPDWLIFAADYSQIELRVLAHIADDDNLIEAFQRDLDIHTKTAMDIFHVSEEEVTANMRRQAKAVNFGIVYGISDYGLAQNLNITRKEAAEFIERYFASFPGVKQYMENIVQEAKQKGYVTTLLHRRRYLPDITSRNFNVRSFAERTAMNTPIQGSAADIIKKAMIDLAARLKEEQLQARLLLQVHDELILEAPKEEIERLCELVPEVMEQAVTLRVPLKVDYHYGPTWYDAK

SEQ ID NO: 2 - protein, 876 aa, Geobacillus stearothermophilus
MKKKLVLIDGNSVAYRAFFALPLLHNDKGIHTNAVYGFTMMLNKILAEEQPTHLLVAFDAGKTTFRHETFQEYKGGRQQTPPELSEQFPLLRELLKAYRIPAYELDHYEADDIIGTLAARAEQEGFEVKIISGDRDLTQLASRHVTVDITKKGITDIEPYTPETVREKYGLTPEQIVDLKGLMGDKSDNIPGVPGIGEKTAVKLLKQFGTVENVLASIDEVKGEKLKENLRQHRDLALLSKQLASICRDAPVELSLDDIVYEGQDREKVIALFKELGFQSFLEKMAAPAAEGEKPLEEMEFAIVDVITEEMLADKAALVVEVMEENYHDAPIVGIALVNEHGRFFMRPETALADSQFLAWLADETKKKSMFDAKRAVVALKWKGIELRGVAFDLLLAAYLLNPAQDAGDIAAVAKMKQYEAVRSDEAVYGKGVKRSLPDEQTLAEHLVRKAAAIWALEQPFMDDLRNNEQDQLLTKLEQPLAAILAEMEFTGVNVDTKRLEQMGSELAEQLRAIEQRIYELAGQEFNINSPKQLGVILFEKLQLPVLKKTKTGYSTSADVLEKLAPHHEIVENILHYRQLGKLQSTYIEGLLKVVRPDTGKVHTMFNQALTQTGRLSSAEPNLQNIPIRLEEGRKIRQAFVPSEPDWLIFAADYSQIELRVLAHIADDDNLIEAFQRDLDIHTKTAMDIFHVSEEEVTANMRRQAKAVNFGIVYGISDYGLAQNLNITRKEAAEFIERYFASFPGVKQYMENIVQEAKQKGYVTTLLHRRRYLPDITSRNFNVRSFAERTAMNTPIQGSAADIIKKAMIDLAARLKEEQLQARLLLQVHDELILEAPKEEIERLCELVPEVMEQAVTLRVPLKVDYHYGPTWYDAK

SEQ ID NO: 3 - DNA, 1764 bp, Geobacillus stearothermophilus
  source 1..1764: mol_type = genomic DNA
gcagaaggggagaaaccgcttgaggagatggagtttgccatcgttgacgtcattaccgaagagatgcttgccgacaaggcagcgcttgtcgttgaggtgatggaagaaaactaccacgatgccccgattgtcggaatcgcactagtgaacgagcatgggcgattttttatgcgcccggagaccgcgctggctgattcgcaatttttagcatggcttgccgatgaaacgaagaaaaaaagcatgtttgacgccaagcgggcagtcgttgccttaaagtggaaaggaattgagcttcgcggcgtcgcctttgatttattgctcgctgcctatttgctcaatccggctcaagatgccggcgatatcgctgcggtggcgaaaatgaaacaatatgaagcggtgcggtcggatgaagcggtctatggcaaaggcgtcaagcggtcgctgccggacgaacagacgcttgctgagcatctcgttcgcaaagcggcagccatttgggcgcttgagcagccgtttatggacgatttgcggaacaacgaacaagatcaattattaacgaagcttgagcagccgctggcggcgattttggctgaaatggaattcactggggtgaacgtggatacaaagcggcttgaacagatgggttcggagctcgccgaacaactgcgtgccatcgagcagcgcatttacgagctagccggccaagagttcaacattaactcaccaaaacagctcggagtcattttatttgaaaagctgcagctaccggtgctgaagaagacgaaaacaggctattcgacttcggctgatgtgcttgagaagcttgcgccgcatcatgaaatcgtcgaaaacattttgcattaccgccagcttggcaaactgcaatcaacgtatattgaaggattgttgaaagttgtgcgccctgataccggcaaagtgcatacgatgttcaaccaagcgctgacgcaaactgggcggctcagctcggccgagccgaacttgcaaaacattccgattcggctcgaagaggggcggaaaatccgccaagcgttcgtcccgtcagagccggactggctcattttcgccgccgattactcacaaattgaattgcgcgtcctcgcccatatcgccgatgacgacaatctaattgaagcgttccaacgcgatttggatattcacacaaaaacggcgatggacattttccatgtgagcgaagaggaagtcacggccaacatgcgccgccaggcaaaggccgttaacttcggtatcgtttacggaattagcgattacggattggcgcaaaacttgaacattacgcgcaaagaagctgccgaatttatcgaacgttacttcgccagctttccgggcgtaaagcagtatatggaaaacattgtgcaagaagcgaaacagaaaggatatgtgacaacgctgttgcatcggcgccgctatttgcctgatattacaagccgcaatttcaacgtccgcagttttgcagagcggacggccatgaacacgccaattcaaggaagcgccgctgacattattaaaaaagcgatgattgatttagcggcacggctgaaagaagagcagcttcaggctcgtcttttgctgcaagtgcatgacgagctcattttggaagcgccaaaagaggaaattgagcgattatgtgagcttgttccggaagtgatggagcaggccgttacgctccgcgtgccgctgaaagtcgactaccattacggcccaacatggtatgatgccaaataa

SEQ ID NO: 4 - DNA, 41 bp, synthetic construct
  source 1..41: mol_type = other DNA
ggagttctcaatggtggcaccaactactacacgaccatcca

SEQ ID NO: 5 - DNA, 41 bp, synthetic construct
  source 1..41: mol_type = other DNA
gtcctgcagatcgacaacgcctccgtctcaaacttggttcg

SEQ ID NO: 6 - DNA, 18 bp, synthetic construct
  source 1..18: mol_type = other DNA
tggtaccagaagcagggg

SEQ ID NO: 7 - DNA, 19 bp, synthetic construct
  source 1..19: mol_type = other DNA
gttgatgtcggcctccacg

SEQ ID NO: 8 - DNA, 18 bp, synthetic construct
  source 1..18: mol_type = other DNA
agaatcttgtcccgcagg

SEQ ID NO: 9 - DNA, 17 bp, synthetic construct
  source 1..17: mol_type = other DNA
cgtctggctgcagatga